European Patent Application EP 4 324 842 A1, published February 21, 2024. Title: Signal sequences for inducing secretion of proteins in intestinal microorganism. Applicant: Korea Research Institute of Bioscience and Biotechnology. The sequence listing filed with the application follows.

SEQUENCE LISTING (10 sequences)

SEQ ID NO: 1 - protein, 25 aa, Artificial Sequence
  Bt3742 amino acid sequence
MKIMKKRLLYLFMLICSISLFVSCS

SEQ ID NO: 2 - protein, 23 aa, Artificial Sequence
  Bt4368 amino acid sequence
MKIKTLVAMLFLSAGATTVVAQD

SEQ ID NO: 3 - protein, 24 aa, Artificial Sequence
  1102ss amino acid sequence
MKSILNTITAMLAAVLFVPAASAQ

SEQ ID NO: 4 - protein, 22 aa, Artificial Sequence
  pelB amino acid sequence
MKYLLPTAAAGLLLLAAQPAMA

SEQ ID NO: 5 - protein, 118 aa, Artificial Sequence
  YebF amino acid sequence
MKKRGAFLGLLLVSACASVFAANNETSKSVTFPKCEDLDAAGIAASVKRDYQQNRVARWADDQKIVGQADPVAWVSLQDIQGKDDKWSVPLTVRGKSADIHYQVSVDCKAGMAEYQRR

SEQ ID NO: 6 - DNA, 75 bp, Artificial Sequence
  Bt3742 DNA sequence
atgaagattatgaagaaaagattgttgtatttgttcatgcttatttgttccataagtttatttgtgagttgtagt

SEQ ID NO: 7 - DNA, 69 bp, Artificial Sequence
  Bt4368 DNA sequence
atgaaaattaaaacgcttgtggctatgttgttcctttcggctggagcaaccactgtggtggcacaggat

SEQ ID NO: 8 - DNA, 72 bp, Artificial Sequence
  1102ss DNA sequence
atgaagtcaatccttaacacaatcacagctatgcttgcggctgttctgttcgtaccggctgcatctgcccag

SEQ ID NO: 9 - DNA, 66 bp, Artificial Sequence
  pelB DNA sequence
atgaaatacctgctgccgaccgctgctgctggtctgctgctcctcgctgcccagccggcgatggcc

SEQ ID NO: 10 - DNA, 354 bp, Artificial Sequence
  YebF DNA sequence
atgaaaaaaagaggggcgtttttagggctgttgttggtttctgcctgcgcatcagttttcgctgccaataatgaaaccagcaagtcggtcactttcccaaagtgtgaagatctggatgctgccggaattgccgcgagcgtaaaacgtgattatcaacaaaatcgcgtggcgcgttgggcagatgatcaaaaaattgtcggtcaggccgatcccgtggcttgggtcagtttgcaggacattcagggtaaagatgataaatggtcagtaccgctaaccgtgcgtggtaaaagtgccgatattcattaccaggtcagcgtggactgcaaagcgggaatggcggaatatcagcggcgt